European Patent Application EP 4 520 822 A1, published March 12, 2025. Title: Kit for pathological condition judgment of Rett syndrome and use of gene contained in mitochondrial genome as biomarker. Applicant: INSTITUTE OF RHEOLOGICAL FUNCTION OF FOOD CO., LTD. Application WO. The sequence listing filed with the application follows.

SEQUENCE LISTING (32 sequences)

SEQ ID NO: 1 - DNA, 33 bp, synthetic construct
  source 1..33: mol_type = other DNA
gacgaggtaccggtgaattctagatcttgagac

SEQ ID NO: 2 - DNA, 33 bp, synthetic construct
  source 1..33: mol_type = other DNA
gtctcaagatctagaattcaccggtacctcgtc

SEQ ID NO: 3 - DNA, 24 bp, synthetic construct
  source 1..24: mol_type = other DNA
gccagcctctcctgattttagtgt

SEQ ID NO: 4 - DNA, 24 bp, synthetic construct
  source 1..24: mol_type = other DNA
gggaacacaaaagacctcttctgg

SEQ ID NO: 5 - DNA, 22 bp, synthetic construct
  source 1..22: mol_type = other DNA
ccgcaagggaaagatgaaagac

SEQ ID NO: 6 - DNA, 20 bp, synthetic construct
  source 1..20: mol_type = other DNA
tcgtttggtttcggggtttc

SEQ ID NO: 7 - DNA, 20 bp, synthetic construct
  source 1..20: mol_type = other DNA
cagaccgcaacctaaacaca

SEQ ID NO: 8 - DNA, 19 bp, synthetic construct
  source 1..19: mol_type = other DNA
ttctgggtgcccaaagaat

SEQ ID NO: 9 - DNA, 20 bp, synthetic construct
  source 1..20: mol_type = other DNA
accgagtcgttctgccaata

SEQ ID NO: 10 - DNA, 20 bp, synthetic construct
  source 1..20: mol_type = other DNA
gcttgatttagtcggcctgg

SEQ ID NO: 11 - DNA, 20 bp, synthetic construct
  source 1..20: mol_type = other DNA
aggccaccacactcctattg

SEQ ID NO: 12 - DNA, 20 bp, synthetic construct
  source 1..20: mol_type = other DNA
gaggtcagcagcctcctaga

SEQ ID NO: 13 - DNA, 20 bp, synthetic construct
  source 1..20: mol_type = other DNA
gttcgcagtcatagccacag

SEQ ID NO: 14 - DNA, 20 bp, synthetic construct
  source 1..20: mol_type = other DNA
gggatggctgataggaggtt

SEQ ID NO: 15 - DNA, 20 bp, synthetic construct
  source 1..20: mol_type = other DNA
cagcctgacccatagccata

SEQ ID NO: 16 - DNA, 20 bp, synthetic construct
  source 1..20: mol_type = other DNA
aagaataacgcgaatgggcc

SEQ ID NO: 17 - DNA, 20 bp, synthetic construct
  source 1..20: mol_type = other DNA
ggatcccactgcacatagga

SEQ ID NO: 18 - DNA, 20 bp, synthetic construct
  source 1..20: mol_type = other DNA
gtcctcctcatgcccctatg

SEQ ID NO: 19 - DNA, 22 bp, synthetic construct
  source 1..22: mol_type = other DNA
tctagttgcattctgactcccc

SEQ ID NO: 20 - DNA, 20 bp, synthetic construct
  source 1..20: mol_type = other DNA
gaatggtagacgtgcagagc

SEQ ID NO: 21 - DNA, 20 bp, synthetic construct
  source 1..20: mol_type = other DNA
ccactgctaattgccctcat

SEQ ID NO: 22 - DNA, 20 bp, synthetic construct
  source 1..20: mol_type = other DNA
tgctattatgcatgccaacc

SEQ ID NO: 23 - DNA, 22 bp, synthetic construct
  source 1..22: mol_type = other DNA
tcgctctcacctaatatccaca

SEQ ID NO: 24 - DNA, 20 bp, synthetic construct
  source 1..20: mol_type = other DNA
ggctgcgaaaactaagatgg

SEQ ID NO: 25 - DNA, 20 bp, synthetic construct
  source 1..20: mol_type = other DNA
tcctactggtccgattccac

SEQ ID NO: 26 - DNA, 20 bp, synthetic construct
  source 1..20: mol_type = other DNA
tttgatgtcgttttgggtga

SEQ ID NO: 27 - DNA, 20 bp, synthetic construct
  source 1..20: mol_type = other DNA
ttggttgtcttgggttagca

SEQ ID NO: 28 - DNA, 20 bp, synthetic construct
  source 1..20: mol_type = other DNA
cgatccaccaaaccctaaaa

SEQ ID NO: 29 - DNA, 20 bp, synthetic construct
  source 1..20: mol_type = other DNA
tcccatcctcaaaacgccta

SEQ ID NO: 30 - DNA, 20 bp, synthetic construct
  source 1..20: mol_type = other DNA
agggttcatgtccgtccttt

SEQ ID NO: 31 - DNA, 19 bp, synthetic construct
  source 1..19: mol_type = other DNA
aacattcccactggcacct

SEQ ID NO: 32 - DNA, 20 bp, synthetic construct
  source 1..20: mol_type = other DNA
ggggtaatgaatgaggcaaa